European Patent Specification EP 3 341 495 B9, published October 4, 2023. Title: ZIC1 and GHSR, molecular diagnostic markers for HPV-induced invasive cancers, nonHPV-induced gynaecological and anogenital cancers and their high-grade precursor lesions. Applicant: Self-screen B.V. The sequence listing filed with the application follows.

SEQUENCE LISTING (8 sequences)

SEQ ID NO: 1 - DNA, 19 bp, Artificial Sequence
  primer
gggcgggttaatgagttgc

SEQ ID NO: 2 - DNA, 22 bp, Artificial Sequence
  primer
tcacgtactaccgacgctaacg

SEQ ID NO: 3 - DNA, 19 bp, Artificial Sequence
  probe
cgccgcgccaacgaaaaac

SEQ ID NO: 4 - DNA, 24 bp, Artificial Sequence
  primer
gtttggtttttgcggtttttattc

SEQ ID NO: 5 - DNA, 21 bp, Artificial Sequence
  primer
caaccctacctcgcatttacg

SEQ ID NO: 6 - DNA, 27 bp, Artificial Sequence
  probe
ctcgatccaattccatctcgcacttcc

SEQ ID NO: 7 - DNA, 2750 bp, Homo sapiens
gagagacagggttagcgggggcagtcgaaggagacaacggaaaggcagaaaacagaaaaataacgcaagagagagaaaaagtaaaggaaactggcaacaacgtttcaaatttgccattaaaaaattcaaacctcaataacctgggaacttaagcgctttcatccacctgtgtgtgtgagtgtgtgtgtgtgtgtgttttcggggaggggggtgcggtggtgccggaagtctgattagataaaagcgagaaatacagaggctgccggttacactgagaaattacatttttttgtaaagagagcatagtgcccgtgtgctcccaagatcttaaattataaacaggagggggacaaagcaagagggaaacaaacttcaaaaggagcaaataacaaaagcctcttttgctgctcttgaagggaggggggaagggggaagaaagaaaagaaagttgctgaatcgggacattctggaagtgcctttgctgtgtttactagccccatccccgcctgctgcacccggagacgtctgaagtctctaatcgctcagcgaaaagttggtttcgggaagggcagcgccggggtgcgggagggcaaaggaggaagaggaatgcatatgactgtgagaaggaaaagtaatcgtggcaaaaaaaaaaaaaaaaaaaaaaaaagaaagaaagaaaagaaaaaagaaaaaaaatttccgtgagaagagggaaaaaatttggctaaaaaaaaagttgctactcctggcagccctggtttgtcaaaaggggatgtcaagcgctttacaatacctgggattgatgaggcgggcgggccaatgagctgcgcgcggcgcctcggcgcgccctccgttggcgcggcggctgagggcggggggaatgcgggcgcaccaatgggcgccagcgtcggcagcacgtgacacctcccccctgctcccattcatcaagggggggacggtgtcgtcctttcaattcatttatctgcaggaatgattgctgctatcagtctcgcgctcaccgcccggctgaggaggtgaaagtttctccccaggaagataaaccgcaaaagacaatattgtgcatgatttgcgccttttctttggctttttctttctttcttcacccccccacccacttttttttttttttttttcaaaaagcagagagggaaaaacggagagtgaaggagcgaggaggcgagcgtgagagaaaggagagagagagaaaagaaagggcgaggggctagtggagaagtaaggaggggcgcgctgcgcgaggcggagagagggcgaagcagtcgcggcactggcgctcacattcctctatgctacaaatccaggaggaagtttttttttagggggctgagatgctccatgcctttccccgggcagccttgacgcgcggccctctcggcagagactgagcggcgagaaagtgcgagccgggccggcagaatctgcctggcgggcgctggagcctgcgttactcgcggcccgcagccgtccggctactttgcgtttggcccggccagcgcccgggcgcgccgcgccattgcctgcaggctaggacttcgcgaggtgggtcgactccccctccctcctcctcttcttcctcctcttcctcctcctcttgttcctcctcctcctcccgattttccctcctcggctggcgagggtggggggggcgggggaggccggggctcgccccgagcagccacgatgctcctggacgccggcccccagtacccagcgatcggcgtgaccacctttggcgcgtcccgccaccactccgcgggcgacgtggccgaacgagacgtgggcctgggcatcaacccgttcgccgacggcatgggcgccttcaagctcaaccccagttcgcacgagctggcttcggccggccagacggccttcacgtcgcaggcgccaggctacgcggctgctgcggccctgggccatcaccatcacccgggccacgtcggctcctattccagcgcagccttcaactccacgcgggactttctgttccgcaaccggggttttggcgacgcggcggcggcagccagcgcacagcacagcctctttgctgcatcggccgggggcttcgggggcccacacggccacacggacgccgcgggccacctcctcttccccgggcttcacgagcaggctgccggccacgcgtcgcctaacgtggtcaacgggcagatgaggctcggcttctcgggggacatgtacccgcgaccggagcagtacggccaggtgaccagcccgcgttcggagcactatgctgcgccgcagctgcacggctacgggcccatgaacgtgaacatggccgcgcatcacggcgccggcgccttcttccgctacatgcgccaacccatcaagcaagagctcatctgcaagtggatcgagcccgagcagctggccaaccccaaaaagtcgtgcaacaaaactttcagcaccatgcacgagctagttacgcacgtcaccgtggagcacgtaggtggcccggagcagagtaatcacatctgcttctgggaggagtgtccgcgcgagggcaagcccttcaaagccaaatacaaactggttaaccacatccgcgtgcacacgggcgagaagccctttccctgccccttccctggctgtggcaaggtcttcgcgcgctccgagaatttaaagatccacaaaaggacgcacacaggggagaagcccttcaagtgcgagtttgagggctgtgaccggcgcttcgc

SEQ ID NO: 8 - DNA, 2144 bp, Homo sapiens
cagcctcacagcctcttcttcacttgccgcctccacacacctccaaccctgcctttttcctttctcctgttccctccctgaccaacctcggcaccccgccaccaggtttgcatcaagcaaaagtaatataccctacagcagactctctaccactaccgagtgatacaaaggactgggattctggacagggtttactcacatatcttgcccctgtgcgctcagaagtcccaaccgggtgggagatccgacactggtccccgagtccccagctcgctgtgtgaccttggacaagtagtcacatcgctgaacctgggtcctataactgcgtgagactattctttggtgctcaccggtatgaatacaaacacaaggtccttcttttctctctctatcccccttcccaagtcgagttggtcaagctcgctttttctttccaccagggccatagccagctgcagccttgtggaggaagaaatcaggtcccagctgctaaaggtgtcctccccaccgccaccgtcgtcttcacccccacccccgggtgtgacctgtccttccggggcacactagtccagcgtcgcccagggcttcggagagagcgcctcacgctcccgcttcgcggcgcctggtccctgcggtccccactcgctgcgacgctttgggaagtgcgagatggaactggatcgagaacgcaaatgcgaggcagggctggtgacaggtatgcgtgtgggcgccggccggaggatgtgttgggagaaactttgggggagttggtgggggaaaggggaggtgtcagagaaagcagtgggtcactctctcacccactgaccaccagtctctctccctcttccttgtccccatctcaccttcttcctcggcttctgcctctcacctccctctctttcttctccaagcatcctccctacgcgtctgcacccgctcctccctcgcaccctcccgcgcctaagcggacctcctcgggagccagctcggtccagcctcccagcgcagtcacgtcccagagcctgttcagctgagccggcagcatgtggaacgcgacgcccagcgaagagccggggttcaacctcacactggccgacctggactgggatgcttcccccggcaacgactcgctgggcgacgagctgctgcagctcttccccgcgccgctgctggcgggcgtcacagccacctgcgtggcactcttcgtggtgggcatcgctggcaacctgctcaccatgctggtggtgtcgcgcttccgcgagctgcgcaccaccaccaacctctacctgtccagcatggccttctccgatctgctcatcttcctctgcatgcccctggacctcgttcgcctctggcagtaccggccctggaacttcggcgacctcctctgcaaactcttccaattcgtcagtgagagctgcacctacgccacggtgctcaccatcacagcgctgagcgtcgagcgctacttcgccatctgcttcccactccgggccaaggtggtggtcaccaaggggcgggtgaagctggtcatcttcgtcatctgggccgtggccttctgcagcgccgggcccatcttcgtgctagtcggggtggagcacgagaacggcaccgacccttgggacaccaacgagtgccgccccaccgagtttgcggtgcgctctggactgctcacggtcatggtgtgggtgtccagcatcttcttcttccttcctgtcttctgtctcacggtcctctacagtctcatcggcaggaagctgtggcggaggaggcgcggcgatgctgtcgtgggtgcctcgctcagggaccagaaccacaagcaaaccgtgaaaatgctggctgtagtggtgtttgccttcatcctctgctggctccccttccacgtagggcgatatttattttccaaatcctttgagcctggctccttggagattgctcagatcagccagtactgcaacctcgtgtcctttgtcctcttctacctcagtgctgccatcaaccccattctgtacaacatcatgtccaagaagtaccgggtggcagtgttcagacttctgggattcgaacccttctcccagagaaagctctccactctgaaagatgaaagttctcgggcctggacagaatctagtattaatacatga